European Patent Specification EP 3 607 036 B1, published February 7, 2024. Title: Detergent compositions comprising Bacterial mannanases. Applicant: Henkel AG & Co. KGaA. The sequence listing filed with the application follows.

SEQUENCE LISTING (48 sequences)

SEQ ID NO: 1 - DNA, 39 bp, Artificial Sequence
  primer
caaccgcctctgcagcttatgcacaaaacggatttcacg

SEQ ID NO: 2 - DNA, 39 bp, Artificial Sequence
  primer
cggtatatctctgtcttaatcactcttaagcccattttc

SEQ ID NO: 3 - DNA, 37 bp, Artificial Sequence
  primer
caaccgcctctgcagcttctgatggtcatagccaaac

SEQ ID NO: 4 - DNA, 36 bp, Artificial Sequence
  primer
cggtatatctctgtcttattggattgttacatgatc

SEQ ID NO: 5 - DNA, 40 bp, Artificial Sequence
  primer
caaccgcctctgcagctgcaagcgggttttatgtaaacgg

SEQ ID NO: 6 - DNA, 39 bp, Artificial Sequence
  primer
cggtatatctctgtcttatttaatggtaacgttatcaac

SEQ ID NO: 7 - DNA, 17 bp, Artificial Sequence
  primer
agctgcagaggcggttg

SEQ ID NO: 8 - DNA, 21 bp, Artificial Sequence
  primer
gacagagatataccgacagtg

SEQ ID NO: 9 - DNA, 975 bp, Bacillus clausii
atgaagagggaggacatggatcaaatgaaaagaaagcggttacaattgtttggaacactagtggtattggttttgttcgtgtacggtagcggttcggcatatgcacaaaacggatttcacgtatccggtacagagttgttggacaaaaatggcgatccttatgttatgcgtggcgtcaaccatggacactcttggtttaagcaagatctggaggaagcaatccctgccatagcagaaacaggggcgaacacggtgagaatggtcttatccaatggacagcaatgggaaaaagatgatgcctctgagcttgcccgtgtgctggctgccacagaaacatatggattgacaactgtgctggaagtccatgacgctacaggaagtgacgatcctgctgatttagagaaagcagtcgattattggatcgaaatggctgatgttctcaaggggacagaagaccgagtaatcattaacgttgccaatgaatggtatgggtcgtggaggagcgacgtttgggcagaagcatacgcacaagcgatcccgcgcttgcgcagcgctggcctctcccatacattaatggttgatgcggcaggttggggccagtaccctgcctccatccacgagcggggagccgatgtgtttgcgtccgatccattaaaaaacacgatgttttcgatccatatgtacgaatatgcaggagctgatagggcgacaattgcctataacattgatcgtgtgcttgctgaaaatcttgctgtggtgatcggtgaatttggccataggcatcatgatggcgatgtcgatgaagatgcgattttggcctatacagcagagcggcaagtgggctggctggcctggtcatggtatggcaacagcgggggtgttgaatacttggatttagctgaaggcccatcaggcccattgacgagttggggcaaacgaattgtttatggtgaaaatgggcttaagagtgattaa

SEQ ID NO: 10 - DNA, 870 bp, Bacillus clausii
cagaacggcttccacgtctccggcacggagctcctggacaagaacggcgacccttacgtcatgcgcggcgtcaaccacggccacagctggttcaagcaggacctcgaggaagccatccctgctatcgctgagacgggcgctaacacggtccgcatggtcctgagcaacggccagcagtgggagaaggacgacgctagcgagctggctcgcgtcctcgctgctacggagacgtacggcctcaccacggtcctggaggtccacgacgctacgggctcggacgaccccgccgacctcgagaaggccgtcgactactggatcgagatggctgacgtcctgaagggcaccgaggaccgcgtcatcatcaacgtcgccaacgagtggtacggctcctggcgcagcgacgtctgggccgaggcctacgctcaggctatccctcgcctccgctcggccggcctctcccacacgctcatggtcgacgctgccggctggggccagtaccctgcttccatccacgagcgcggcgctgacgtctttgcttcggaccccctgaagaacaccatgttctccatccacatgtacgagtacgctggcgctgaccgcgctaccatcgcctacaacatcgaccgcgtcctggctgagaacctggctgtcgtcatcggcgagtttggccaccgccaccacgacggcgacgtcgacgaggacgctatcctggcttacaccgccgagcgccaggtcggctggctggcttggtcgtggtacggcaactcgggcggcgtcgagtacctggacctggctgagggcccttcgggccctctcacgagctggggcaagcgcatcgtctacggcgagaacggcctgaagagcgactaa

SEQ ID NO: 11 - protein, 324 aa, Bacillus clausii
MKREDMDQMKRKRLQLFGTLVVLVLFVYGSGSAYAQNGFHVSGTELLDKNGDPYVMRGVNHGHSWFKQDLEEAIPAIAETGANTVRMVLSNGQQWEKDDASELARVLAATETYGLTTVLEVHDATGSDDPADLEKAVDYWIEMADVLKGTEDRVIINVANEWYGSWRSDVWAEAYAQAIPRLRSAGLSHTLMVDAAGWGQYPASIHERGADVFASDPLKNTMFSIHMYEYAGADRATIAYNIDRVLAENLAVVIGEFGHRHHDGDVDEDAILAYTAERQVGWLAWSWYGNSGGVEYLDLAEGPSGPLTSWGKRIVYGENGLKSD

SEQ ID NO: 12 - protein, 289 aa, Bacillus clausii
QNGFHVSGTELLDKNGDPYVMRGVNHGHSWFKQDLEEAIPAIAETGANTVRMVLSNGQQWEKDDASELARVLAATETYGLTTVLEVHDATGSDDPADLEKAVDYWIEMADVLKGTEDRVIINVANEWYGSWRSDVWAEAYAQAIPRLRSAGLSHTLMVDAAGWGQYPASIHERGADVFASDPLKNTMFSIHMYEYAGADRATIAYNIDRVLAENLAVVIGEFGHRHHDGDVDEDAILAYTAERQVGWLAWSWYGNSGGVEYLDLAEGPSGPLTSWGKRIVYGENGLKSD

SEQ ID NO: 13 - DNA, 1473 bp, Bacillus hemicellulosilyticus
atgagaaatttcggtaagttaattgtcagttcttgtcttctattcagtttttttctttttgcctctgatggtcatagccaaacacattctggtttttatatcgaaggttcaaccctttatgacgccaacggagagccctttgtaatgagaggtatcaatcatggacatgcctggtataaacatgattctaacgtcgctataccagctattgctaatcaaggagcaaatacaattcgtattgttctgtcagatggtggtcaatgggcaaaagatgatataaacacattaaatcaagtgctcgatttagcagaggaacatgagatgattgctgttgttgaggttcacgatgcaacaggatctaattctatggctgacttaaatcgtgctgtcgattattggattgaaatgaaagacgctttaattggaaaagaagatcgcgtcataattaacattgccaatgaatggtatggagcatgggacggacaaggctgggcaaatggctataaggaggttattccacgtttacgaaatgctggcttcactcatacattaatggtagatgcagctggttggggacaataccctcaatcgattcatgattatggtcaagaggtatttaatgctgatcctttagcaaatacgatgttttccatccatatgtatgaatatgctggcggaaatgcttcaatggtacaatctaatatcgatggtgtcgtcgatcaagggttagctcttgtaataggagaatttgggcatatgcatacggacggagatgttgatgaagcaacgatattgagctactcgcaacaaagaggagtcggttggctagcttggtcttggaaaggcaatgggactcaatgggaatatctagatttatcttatgattggcaaggaacaaacttaacttcttggggaaataccattgtccacgggcctaatggattactcgaaacatccattccaagctcgattttccataccgctccaaacaatggagatccccctcctcataacggtaatgaaacgatcttatatgatttcgaacatggcactcaaggctggtcaggttcttcacttcttggaggaccttggacgacgaatgaatggagtacaaatggtaaccattcattaaaggccgatattttcttatcagctaactccaaacatgaattagcaaaagttgaaaatcgaaatttatcaggctactctactttacaagccactgtccgccatgcacattggggaaatgttggtaatttaacggcgagaatgtatgtaaaaacgggctcaaactatagctggtttaatggtgatcctatcccagtaaactcagcaaatggtacgactgtcactttgcctctttcatctattccaaacctaaatgacgtaaaagaaattggcgttgaatttattggagcttcaaatagcaatggacaaaccgccatttatttagatcatgtaacaatccaataa

SEQ ID NO: 14 - DNA, 1395 bp, Bacillus hemicellulosilyticus
cagacccactcgggcttctacatcgagggctcgacgctctacgacgctaacggcgagccttttgtcatgcgcggcatcaaccacggccacgcctggtacaagcacgactccaacgtcgctatccctgctatcgctaaccagggcgctaacaccatccgcatcgtcctcagcgacggtggccagtgggccaaggacgacatcaacacgctgaaccaggtcctcgacctggccgaggagcacgagatgatcgctgtcgtcgaggtccacgacgctaccggctccaacagcatggccgacctcaaccgcgccgtcgactactggatcgagatgaaggacgccctgatcggcaaggaagaccgcgtcatcatcaacatcgctaacgagtggtacggcgcttgggacggccagggctgggccaacggctacaaggaagtcatccctcgcctgcgcaacgctggcttcacccacaccctcatggtcgacgctgccggctggggccagtaccctcagagcatccacgactacggccaagaggtcttcaacgccgaccctctggccaacaccatgttctccatccacatgtacgagtacgctggcggcaacgcctccatggtccagagcaacatcgacggcgtcgtcgaccagggcctcgctctggtcatcggcgagttcggccacatgcacacggacggcgacgtcgacgaggctaccatcctgagctactcgcagcagcgcggcgtcggctggctggcctggtcgtggaagggcaacggcacccagtgggagtacctcgacctgagctacgactggcagggcaccaacctcacgtcgtggggcaacacgatcgtccacggccctaacggcctcctggagacgtccatcccttccagcatctttcacaccgctcctaacaacggcgaccctcctccccacaacggcaacgagacgatcctgtacgacttcgagcacggcacgcagggctggtcgggctcgtccctgctgggcggcccttggaccaccaacgagtggtcgaccaacggcaaccactccctcaaggccgacatcttcctgtccgccaacagcaagcacgagctcgccaaggtcgagaaccgcaacctcagcggctactcgacgctgcaggctaccgtccgccacgctcactggggcaacgtcggcaacctgacggctcgcatgtacgtcaagacgggcagcaactactcgtggttcaacggcgaccccatccctgtcaactcggctaacggcaccaccgtcaccctccctctgagctcgatccccaacctcaacgacgtcaaggagatcggcgtcgagttcatcggcgctagcaacagcaacggccagaccgccatctacctggaccacgtcacgatccagtaa

SEQ ID NO: 15 - protein, 490 aa, Bacillus hemicellulosilyticus
MRNFGKLIVSSCLLFSFFLFASDGHSQTHSGFYIEGSTLYDANGEPFVMRGINHGHAWYKHDSNVAIPAIANQGANTIRIVLSDGGQWAKDDINTLNQVLDLAEEHEMIAVVEVHDATGSNSMADLNRAVDYWIEMKDALIGKEDRVIINIANEWYGAWDGQGWANGYKEVIPRLRNAGFTHTLMVDAAGWGQYPQSIHDYGQEVFNADPLANTMFSIHMYEYAGGNASMVQSNIDGVVDQGLALVIGEFGHMHTDGDVDEATILSYSQQRGVGWLAWSWKGNGTQWEYLDLSYDWQGTNLTSWGNTIVHGPNGLLETSIPSSIFHTAPNNGDPPPHNGNETILYDFEHGTQGWSGSSLLGGPWTTNEWSTNGNHSLKADIFLSANSKHELAKVENRNLSGYSTLQATVRHAHWGNVGNLTARMYVKTGSNYSWFNGDPIPVNSANGTTVTLPLSSIPNLNDVKEIGVEFIGASNSNGQTAIYLDHVTIQ

SEQ ID NO: 16 - protein, 464 aa, Bacillus hemicellulosilyticus
QTHSGFYIEGSTLYDANGEPFVMRGINHGHAWYKHDSNVAIPAIANQGANTIRIVLSDGGQWAKDDINTLNQVLDLAEEHEMIAVVEVHDATGSNSMADLNRAVDYWIEMKDALIGKEDRVIINIANEWYGAWDGQGWANGYKEVIPRLRNAGFTHTLMVDAAGWGQYPQSIHDYGQEVFNADPLANTMFSIHMYEYAGGNASMVQSNIDGVVDQGLALVIGEFGHMHTDGDVDEATILSYSQQRGVGWLAWSWKGNGTQWEYLDLSYDWQGTNLTSWGNTIVHGPNGLLETSIPSSIFHTAPNNGDPPPHNGNETILYDFEHGTQGWSGSSLLGGPWTTNEWSTNGNHSLKADIFLSANSKHELAKVENRNLSGYSTLQATVRHAHWGNVGNLTARMYVKTGSNYSWFNGDPIPVNSANGTTVTLPLSSIPNLNDVKEIGVEFIGASNSNGQTAIYLDHVTIQ

SEQ ID NO: 17 - DNA, 1449 bp, Virgibacillus soli
atgttattctctacttcactgtttacttctacttcaaaagcgaatgcagcaagcgggttttatgtaaacggaaacacactctatgacgcaacaggtaccccttttgtgataagaggaatcaatcatgctcactcttggtttaaagacgacacagcaaccgcaatacctgccattgcagcaactggggcgaatactattagaatcgtattatcggatggcagccaatatagtcgggatgatattgatggcgtgaggaatctaatatcattggctgaggaaaataatctaattgctatgttagaggtccacgatgctactggaaaagatgatatcagctcattagatagtgcggcagattattggattagtataaaagaagcacttatcggcaaggaagacaaagtcctaataaacatcgcaaatgaatggtacggtacttgggatggggctagttgggcggatggctacaaacaagtgattcccaaattaagaaatgcaggacttaaccacacactaatagtagactctgctggctgggggcaatttccggagtccattcacaattacggaaaagaagtattcaatgctgaccccctacaaaatacaatgttctctattcatatgtatgaatatgctggtggggacgcttctactgtcaaagcaaatattgacggtgtattaaatcaaggtctagccgtaatcattggagaatttggacataggcatacagacggagatgtagatgaagcaacaattatgaattattcccaagagaaaaatgttggctggctcgcatggtcgtggaaaggtaatggcatggaatgggattatttagacttatcctatgattgggccggaaataacctaaccgactggggaaataccattgtaaatagtacaaacggcttaaaagctacatctgaaataagtccagtatttggagatggagatgacggtgtaggcgacggtggtcctggggattctaacggaactgaaactacgctttataacttcgaaaccgggacagaaggatggagcggcgaaaatatagaaactggaccttggtcagtgaatgagtgggcagcaaaaggtaaccactctttaaaagctgatgttaatttgggtgataactctgaacattatctatacctaactcaaaacctaaattttagcggaaagtcacaactcacagcgactgtaaagcatgctgattggggaaacttcggggatgaaataaatgcaaagttatatgtaaaaacagaatcagattggcaatggtttgatggaggaattgaaaagatcaattcttcaattggaactattataaccttagatttatcatcgctctcaaacccaagtgatattaaagaagttggtgttcagtttacgggttcttcaaatagttatggcctaacagctttatatgttgataacgttaccattaaataa

SEQ ID NO: 18 - DNA, 1401 bp, Virgibacillus soli
gcctcgggcttctacgtcaacggcaacactctctacgacgccacgggcaccccatttgtcatccgcggcatcaaccacgctcactcgtggttcaaggacgacactgccaccgctatccctgctatcgctgctacgggcgccaacacgatccgcatcgtcctcagcgacggctcgcagtactcccgcgacgacatcgacggcgtccgcaacctcatctccctggccgaggagaacaacctcatcgccatgctggaggtccacgacgctaccggcaaggacgacatcagctcgctggacagcgccgccgactactggatctcgatcaaggaagccctcatcggcaaggaagacaaggtcctgatcaacatcgccaacgagtggtacggcacctgggacggcgctagctgggctgacggctacaagcaggtcatccctaagctccgcaacgccggcctcaaccacacgctcatcgtcgactcggctggctggggccagttcccggagagcatccacaactacggcaaggaagtcttcaacgccgaccccctgcagaacacgatgttctcgatccacatgtacgagtacgccggcggcgacgcttccacggtcaaggccaacatcgacggcgtcctcaaccagggcctggctgtcatcatcggcgagtttggccaccgccacaccgacggcgacgtcgacgaggccaccatcatgaactacagccaggagaagaacgtcggctggctggcttggagctggaagggcaacggcatggagtgggactacctcgacctgagctacgactgggccggcaacaacctcaccgactggggcaacacgatcgtcaactcgaccaacggcctgaaggccacctcggagatcagccctgtctttggcgacggcgacgacggcgtcggcgacggtggccccggcgacagcaacggcaccgagacgacgctgtacaactttgagacgggcaccgagggctggagcggcgagaacatcgagacgggcccttggtcggtcaacgagtgggctgccaagggcaaccactccctcaaggccgacgtcaacctgggcgacaacagcgagcactacctctacctgacgcagaacctcaacttctccggcaagtcgcagctgacggctaccgtcaagcacgctgactggggcaacttcggcgacgagatcaacgccaagctctacgtcaagaccgagagcgactggcagtggttcgacggtggcatcgagaagatcaactccagcatcggcaccatcatcacgctcgacctgtcgtccctgtcgaacccgtccgacatcaaggaagtcggcgtccagttcactggctcgtctaactcttacggcctcactgctctttacgtcgacaacgtcactatcaagtag

SEQ ID NO: 19 - protein, 482 aa, Virgibacillus soli
MLFSTSLFTSTSKANAASGFYVNGNTLYDATGTPFVIRGINHAHSWFKDDTATAIPAIAATGANTIRIVLSDGSQYSRDDIDGVRNLISLAEENNLIAMLEVHDATGKDDISSLDSAADYWISIKEALIGKEDKVLINIANEWYGTWDGASWADGYKQVIPKLRNAGLNHTLIVDSAGWGQFPESIHNYGKEVFNADPLQNTMFSIHMYEYAGGDASTVKANIDGVLNQGLAVIIGEFGHRHTDGDVDEATIMNYSQEKNVGWLAWSWKGNGMEWDYLDLSYDWAGNNLTDWGNTIVNSTNGLKATSEISPVFGDGDDGVGDGGPGDSNGTETTLYNFETGTEGWSGENIETGPWSVNEWAAKGNHSLKADVNLGDNSEHYLYLTQNLNFSGKSQLTATVKHADWGNFGDEINAKLYVKTESDWQWFDGGIEKINSSIGTIITLDLSSLSNPSDIKEVGVQFTGSSNSYGLTALYVDNVTIK

SEQ ID NO: 20 - protein, 466 aa, Virgibacillus soli
ASGFYVNGNTLYDATGTPFVIRGINHAHSWFKDDTATAIPAIAATGANTIRIVLSDGSQYSRDDIDGVRNLISLAEENNLIAMLEVHDATGKDDISSLDSAADYWISIKEALIGKEDKVLINIANEWYGTWDGASWADGYKQVIPKLRNAGLNHTLIVDSAGWGQFPESIHNYGKEVFNADPLQNTMFSIHMYEYAGGDASTVKANIDGVLNQGLAVIIGEFGHRHTDGDVDEATIMNYSQEKNVGWLAWSWKGNGMEWDYLDLSYDWAGNNLTDWGNTIVNSTNGLKATSEISPVFGDGDDGVGDGGPGDSNGTETTLYNFETGTEGWSGENIETGPWSVNEWAAKGNHSLKADVNLGDNSEHYLYLTQNLNFSGKSQLTATVKHADWGNFGDEINAKLYVKTESDWQWFDGGIEKINSSIGTIITLDLSSLSNPSDIKEVGVQFTGSSNSYGLTALYVDNVTIK

SEQ ID NO: 21 - DNA, 60 bp, Artificial Sequence
  primer
agtcaatcgcgacaagcgccagacccactcgggcttctacatcgagggctcgacgctcta

SEQ ID NO: 22 - DNA, 46 bp, Artificial Sequence
  primer
cgcgccggatccttactggatcgtgacgtggtccaggtagatggcg

SEQ ID NO: 23 - DNA, 60 bp, Artificial Sequence
  primer
agtcaatcgcgacaagcgccagaacggcttccacgtctccggcacggagctcctggacaa

SEQ ID NO: 24 - DNA, 51 bp, Artificial Sequence
  primer
cgcgccggatccttagtcgctcttcaggccgttctcgccgtagacgatgcg

SEQ ID NO: 25 - DNA, 1846 bp, Bacillus pumilus
atgaaaaaatgggttcaacgggtggcttgttttatgctgctgatcactttatgggcgggttggttcactctgaccgtaaaggcctcctcctatgtgcaaacatctggtacacattttgtattgaacaaccacccattttactttgctggcacaaataattattatttccattacaaatcaaaaaagatggtagatgctgtttttgacgatatgaaggcaatggatttaaaggttattcgtatttggggatttcacgatggtacccctcaagaaaactcagtcttacaatctcgtccaggtgtttatgaagaatccggttttcaaaaactagactatgcgatttataaagcagggcaggaaggaatcaagctggtcataccgctcgtgaacaattgggatgactttggcgggatgaatcaatatgtgaagtggtttcaggcaggatcacatgatcacttttatacagattctcggattaaaacagcttacaaaaactatgtgcgctatgtattagagagaaccaatacgtactcaggtgttcaatataaagatgaccctgctattatgacatgggagctcgccaatgagccgcgcgctcagtcagacccttcgggagatatactagtaaactgggcagatgaaatgagtgcatggatcaaatcaattgactcgaatcatcttgttgctgtaggagacgaagggttctttcgcatgacaggtcatgatgattggttttacagtggaggagaaggtgttgattgggatcgtttgactgctctccctcatattgattatggaacctatcatttatacccggatcactggaatcagtctgctgcatggggagtgaaatggatcaaagatcatatcacccgaggaaacgcaatcggaaaacctgttgtattagaagagtttggctatcaaaatcaagcagcccgtcctgatgtatatgatagctggctgaagacaattgaacagctcggaggcgcaggtagccaattttggattttaacaagcattcaagacgatgattccctctacccggattatgatggttttcgagttttaaaggagagccgggaggcaggaattattcgtgaacacgccaaaagaatgaatgaaaagaactgatgaagaatgcctgtttataaggaacttcatttgcataaaaaaattggatatggtatagtttttatggaaatgctaacgattaccgagacaagagtggggaaacccgctcttttgtattgaacaggcaatttttgtctcgacattattcatccgttttctgctccccctgctcacaataaagcagggtttttatgcagaatgattgataagagcgtttatcgaaagcacaaggaggaagagaatgagcaaaaaagtagtggatatcgtaagcgacatggtgcagccaattttagatggcttacagcttgaactcgttgatgttgaatttgtcaaagagggtcaaaactggttccttcgcgtatttattgactctgataaaggcgtcgatatcgaggagtgtgccaaagtgagcgaagccttgagcgaaaagcttgatgaggcagatccaattagccaaaactactttcttgaagtgtcctctcctggagcggagcgcccattaaagaaaaaagctgattttgaaaaagcacttggaaaaaatgttttcatgaaaacatacgaaccaattgatggtgaaaaggcatttgaaggtgagcttacaagctttgatggtgagattgcaacagtgacagtgaagatcaagacaagaaagaaagagatcaatattccatacgaaaaaattgctaacgcaagattagcagtttcgttcaattaa

SEQ ID NO: 26 - protein, 376 aa, Bacillus pumilus
MKKWVQRVACFMLLITLWAGWFTLTVKASSYVQTSGTHFVLNNHPFYFAGTNNYYFHYKSKKMVDAVFDDMKAMDLKVIRIWGFHDGTPQENSVLQSRPGVYEESGFQKLDYAIYKAGQEGIKLVIPLVNNWDDFGGMNQYVKWFQAGSHDHFYTDSRIKTAYKNYVRYVLERTNTYSGVQYKDDPAIMTWELANEPRAQSDPSGDILVNWADEMSAWIKSIDSNHLVAVGDEGFFRMTGHDDWFYSGGEGVDWDRLTALPHIDYGTYHLYPDHWNQSAAWGVKWIKDHITRGNAIGKPVVLEEFGYQNQAARPDVYDSWLKTIEQLGGAGSQFWILTSIQDDDSLYPDYDGFRVLKESREAGIIREHAKRMNEKN

SEQ ID NO: 27 - DNA, 1083 bp, Bacillus amyloliquefaciens
atgctcaaaaagttcgcagtctgtctgtctatcattttattactcatctcagccgcccgtccgatatcggctcacaccgtttaccctgtcaatcccaatgcccagcagacgacaaaagacgtcatgaactggctggcgcatttgcccaaccgttcagaaaacagggtcatgtccggtgcattcggcgggtacagcgatgtcaccttttcaatgacggaggaaaaccgcttgaaaaacgcgacgggacagtctcccgccatctacggctgtgattatgggagagggtggctggaaacatcggatatcaccgattctatcgactacagctgcaacagcagcctcatttcgtactggaaaagcggcggcctccctcaggtcagcctgcatctcgcaaatccggcctttccatcaggacactataaaacggccatttcaaacagccagtataaaaatatcctgaacccttcaactgttgaaggacggcggcttgaggccttgctcagcaaaatcgccgacggccttactcagctgaaaaatcaaggcgtcaccgttctgttcaggccgctgcatgagatgaacggtgaatggttctggtgggggctgacaggctacaaccaaaaagacactgagagaatctcgctgtacaaagagctttacaagaagatataccgctatatgacagagacaagaggattggataatcttttgtgggtgtattcgcctgatgccaacagagacttcaaaacagacttctacccaggctcatcttatgtggatattaccggactggatgcttacttcaccgacccgtatgcgatatcaggctatgatgaaatgctgtctctgaaaaaaccgtttgcctttgccgagaccggtccgtccggtaatatcggaagctttgattacgctgtttttatcaatgcgatcaggcaaaagtatcccgagacaacctactttttgacatgggatgaacaattaagcccggcagccaatcaaggcgcgcaaagcctttatcaaaacagctggacgctgaacaagggcgaaatgtggaatggcggaaccttgacgccgatcgcggaataa

SEQ ID NO: 28 - protein, 360 aa, Bacillus amyloliquefaciens
MLKKFAVCLSIILLLISAARPISAHTVYPVNPNAQQTTKDVMNWLAHLPNRSENRVMSGAFGGYSDVTFSMTEENRLKNATGQSPAIYGCDYGRGWLETSDITDSIDYSCNSSLISYWKSGGLPQVSLHLANPAFPSGHYKTAISNSQYKNILNPSTVEGRRLEALLSKIADGLTQLKNQGVTVLFRPLHEMNGEWFWWGLTGYNQKDTERISLYKELYKKIYRYMTETRGLDNLLWVYSPDANRDFKTDFYPGSSYVDITGLDAYFTDPYAISGYDEMLSLKKPFAFAETGPSGNIGSFDYAVFINAIRQKYPETTYFLTWDEQLSPAANQGAQSLYQNSWTLNKGEMWNGGTLTPIAE

SEQ ID NO: 29 - DNA, 1494 bp, Amphibacillus xylanus
gtgaagttaactaaactaaaactattgagtagtgtattttttgttgtattaactgtgttaatgttgtttgtccctgggaatattgtgaatgtaaaagctgctaacggcttttatgtaagcgattccaatctgtatgatgcaaatggaaatcaatttgttatgcgtggggttaatcatgcccattcatggtataaggacacgtataccgaggcaattcctgcaattgcggctacaggagcgaatactatccgaattgtattatctgatggagggcaataccaaaaagatgatataaacatagtcagaaatttgattgaaaccgcagaagccaataatttagtcgctgtacttgaggttcatgatgctactgggtcggattcattatcggatttgaaccgggctgtagattattggattgaaattaaagatgcgttaattggtaaagaagatacggtgatcataaacattgtcaatgaatggtatggcacttgggatggtcgtctctgggcagatggttataaacaggcgataccgagattaagagatgctggattaacacatacgttgatgattgatgcagcaggttgggggcaatttcctagctcgatccatcaatatggtagagaagtatttaatgcagatcgtttagggaatacaatgttttcgattcatatgtatgaatatgctggcggtgatgatcaaatggttagagataatattaacggtgtgatcaatcaagacttagctctagtgattggtgaatttggtcattatcacacagatggcgatgttgatgaagatacgattttgagttacgcggagcagacaggtgttggttggttagcatggtcatggaaaggcaatggaactgagtgggagtatcttgatctatcaaatgattggggaggaaattatttaacatcttggggtgacaggattgtaaatggagcaaatggattaagagaaacgagtcaaattgcttctgttttttcaggaaacaatggcgggactcctggaaatggtgaggaagagactcctggtgatgtaagtcatttcgcaaacttcgagaatggtactgaaggttgggaagcaagcaatgtatctggtggaccttgggcaacaaatgaatggagtgctagtggttcatatgctttaaaagccgatgcgcaattagcatctggaagagaacactatttatatcgaatcggtccctttaatttatctgggtcaacattaaacgcaacggtaaggggtgctaattgggggaattatggatctggtatcgacgtgaagctatacgttaagtacggagatggctggacgtggagagatagtggtgtacagacaattagagcgggagaatctattgatctatcactagatttatcaaatgttgatcgctcaaacattagagaagttggtatccagtttattggtggaaatcattcatctggaaaaaccgctttttatgttgatcatgtttattcacattag

SEQ ID NO: 30 - protein, 497 aa, Amphibacillus xylanus
VKLTKLKLLSSVFFVVLTVLMLFVPGNIVNVKAANGFYVSDSNLYDANGNQFVMRGVNHAHSWYKDTYTEAIPAIAATGANTIRIVLSDGGQYQKDDINIVRNLIETAEANNLVAVLEVHDATGSDSLSDLNRAVDYWIEIKDALIGKEDTVIINIVNEWYGTWDGRLWADGYKQAIPRLRDAGLTHTLMIDAAGWGQFPSSIHQYGREVFNADRLGNTMFSIHMYEYAGGDDQMVRDNINGVINQDLALVIGEFGHYHTDGDVDEDTILSYAEQTGVGWLAWSWKGNGTEWEYLDLSNDWGGNYLTSWGDRIVNGANGLRETSQIASVFSGNNGGTPGNGEEETPGDVSHFANFENGTEGWEASNVSGGPWATNEWSASGSYALKADAQLASGREHYLYRIGPFNLSGSTLNATVRGANWGNYGSGIDVKLYVKYGDGWTWRDSGVQTIRAGESIDLSLDLSNVDRSNIREVGIQFIGGNHSSGKTAFYVDHVYSH

SEQ ID NO: 31 - DNA, 1767 bp, Paenibacillus polymyxa
atgaaaaaactactgtcttgtctcatttcgctgtcaatgcttgtgtatatcttaccgacaatgatagtgtccgctaacaatgatggcgtaacgaaccttgctcttgattcaacacctagtgcgcaaagtgatattatttctgatgctgtctacaaaatcacagctcagcattcaggaaaaagccttgaggttgaaggcggttctaaagatgacggcgcgaatgttcaacaatggacagataacgggaaagaacagcagaaatggagagttgtggacgtcggtggcggatattacaagctcatcagtcaatctagcggaaaagcactggatgtggcaggtggtaatacacatgatggtgccaatgtgcaacagtggacggacaacggaaatgctcagcaaaagtggaagatcatcgatgtaggaggaggctattataagttgatctcacaaagctctggaaaggcactcgacgtcgttggtggttatacgcacgacggggccaatgtgcagcaatgggcagacaatggatctgctcaacagcgctggcgtttcacacaaattgatacaaccacggatacgacgccgccaacagcaccaacgaatttacaatcatcatcgaaaacaagtacctctgtaacattgacttggaccacaagcattgataatgtaggtgtgacaggctatgtcatttataatggaacagatttggtcgggacttctacaactacatcttatattgttacaggattaacagcgaacacttcctataacttcactgtcaaagcgaaggatgccgctgggaatatttcagaaccatcaaatgtcttgaaagtcacaacgagttcagattcttctcaaaacacaggtttttatgtgaagggcacaacattatatgatggaaacggtaatccatttgtgatgagaggaatcaatcatgcatacacatggtataaagggcaagaatcagtagcaattcctgcgattgcgaaaacgggtgcaaacaccatccggattgtcttatctgacggacagcagtggacaaaagatgatttaagcgcgcttcaaaatttgattacactcagtgagcaaaacaaacttgtagtgattttagaggtgcacgacggtactggcaatgacaatgccgcagttttaaataaaattgctgattattggattgaaatgaagtcagctttaattgggaaggaaaatacagttattttaaacatcgcaaatgaatggtttggtacatgggatggaaacggctgggcgcagggctacaaatcagtcataccaaagctgcgaaatgcgggcatcaaaaacacgattatggtggatgcggctggatggggacaatatccaaaatcgatttttgattacggaacgcaagtgttcgatgcagatccgctcaagaatacgatgttttccattcatatgtatgaatacgcaggcggcaacgcagaaacagtgaaaagtaatatcgacaacgtcctgaataaaaatcttgcactcatcattggagaatttggaattaaacatacaaacggagatgttgatgaagcaacgatcatgtcatacgcacagcaaaaaggtgttgggtatcttggctggtcatggaaaggaaatggttcaggtcttgaatatttagatatgagtaacgattgggctggcagcagttatacagagcaaggacatgccattatcgaaggaccaaatggcattcgtgcaacatcaaaattatcaaccatttacagcaatgggaaacaataa

SEQ ID NO: 32 - protein, 588 aa, Paenibacillus polymyxa
MKKLLSCLISLSMLVYILPTMIVSANNDGVTNLALDSTPSAQSDIISDAVYKITAQHSGKSLEVEGGSKDDGANVQQWTDNGKEQQKWRVVDVGGGYYKLISQSSGKALDVAGGNTHDGANVQQWTDNGNAQQKWKIIDVGGGYYKLISQSSGKALDVVGGYTHDGANVQQWADNGSAQQRWRFTQIDTTTDTTPPTAPTNLQSSSKTSTSVTLTWTTSIDNVGVTGYVIYNGTDLVGTSTTTSYIVTGLTANTSYNFTVKAKDAAGNISEPSNVLKVTTSSDSSQNTGFYVKGTTLYDGNGNPFVMRGINHAYTWYKGQESVAIPAIAKTGANTIRIVLSDGQQWTKDDLSALQNLITLSEQNKLVVILEVHDGTGNDNAAVLNKIADYWIEMKSALIGKENTVILNIANEWFGTWDGNGWAQGYKSVIPKLRNAGIKNTIMVDAAGWGQYPKSIFDYGTQVFDADPLKNTMFSIHMYEYAGGNAETVKSNIDNVLNKNLALIIGEFGIKHTNGDVDEATIMSYAQQKGVGYLGWSWKGNGSGLEYLDMSNDWAGSSYTEQGHAIIEGPNGIRATSKLSTIYSNGKQ

SEQ ID NO: 33 - DNA, 1470 bp, Bacillus hemicellulosilyticus
atggatatattaagaaagtgtgtacttgtactattggccttactattgttgttacctacgacatcaacggcattttctgaaagcgcttctactaatgagagagtgctaaatttatctgatccgaatgcgacacgctatacgaaggaattgtttgcgtttcttcaagacgtgagtggtgagcaagtgttgttcgggcaacagcatgcaacagatgaagggttgactctgacaggtgaaggaaatcgaattggttcaactgagtcggaggtgaagaatgcagtaggtgattatccagctgtttttgggtgggatacgaacagcttggatggtcgtgaaaagccaggtacagatgtggaaagtcaagagcaacgaattttaaatacagcagaatcgatgaaagtggcacatgaattaggagggatcatcacattaagtatgcatccggataactttgttaccggtcattactatggcgatacggatggtaacgtcgttcaagaaatattgccaggtggctccaagcacaatgaatttaacgcttggctagataatattgctgccctagcacatgaattagttgatgataatggagagcctattccggttatcttccgtccattccatgagcaaacaggttcgtggttttggtggggtgcgagcacaacaactcctgagcaatacaaagcgatttttcgatatacagtcgaatacttaagagatgcaaagggtgttcataactttttatatggattctcccctggtgcgggtcctgctggcgatctagatcgatatttagaaacgtacccaggtgataattatgtcgatatcttaggtattgataattatgatagtaagtcaaatgcggggtcagacgcttggttatctggaatggtaaaagatttagcgatgatctcgaaattagcagaggaaagagggaaggtatcagcctttactgaatttggatacagcgctgaagggatgagtcaaacgggtgatgcgttagattggtatacacgtgtgttaaatgcgataaaagcagatgaagatgcgcgaaacatatcctacatgctaacgtgggctaactttgggtggcctaataatatatttgttccgtatcgtgatgtgaatggggatttaggtggagatcatgagttattacctgactttgtacagttttatgaagatgaatactcagcatttcgtgaagatataaatgaaagtgtttacaatcgtaatgagagttatattgttgcggatcatgagccatttatgtatgttgtttcccctacgacaggtacatatataacaggctcgtctgttgtcttacgagcgaaagtagttaacgatgaggatccgtccgttacgtatcaagtggcgggttctgaagaagtctatgagatgactttagatgaaaatgggtattactctgctgattatattcctactgctcctaagaatggagctctgtag

SEQ ID NO: 34 - protein, 489 aa, Bacillus hemicellulosilyticus
MDILRKCVLVLLALLLLLPTTSTAFSESASTNERVLNLSDPNATRYTKELFAFLQDVSGEQVLFGQQHATDEGLTLTGEGNRIGSTESEVKNAVGDYPAVFGWDTNSLDGREKPGTDVESQEQRILNTAESMKVAHELGGIITLSMHPDNFVTGHYYGDTDGNVVQEILPGGSKHNEFNAWLDNIAALAHELVDDNGEPIPVIFRPFHEQTGSWFWWGASTTTPEQYKAIFRYTVEYLRDAKGVHNFLYGFSPGAGPAGDLDRYLETYPGDNYVDILGIDNYDSKSNAGSDAWLSGMVKDLAMISKLAEERGKVSAFTEFGYSAEGMSQTGDALDWYTRVLNAIKADEDARNISYMLTWANFGWPNNIFVPYRDVNGDLGGDHELLPDFVQFYEDEYSAFREDINESVYNRNESYIVADHEPFMYVVSPTTGTYITGSSVVLRAKVVNDEDPSVTYQVAGSEEVYEMTLDENGYYSADYIPTAPKNGAL

SEQ ID NO: 35 - DNA, 1110 bp, Bacillus alcalophilus
atgagaagtatgaagcttttatttgctatgtttattttagttttttcctcttttacttttaacttagtagttgcgcaagctagtggacatggacaaatgcataaagtaccttgggcaccccaagctgaagcacctggaaaaacggctgagaatggagtctgggataaagttagaaataatcctggaaaagccaatcctccagcaggaaaagtcaatggtttttatatagatggaacaaccttatatgatgcaaatggtaagccatttgtgatgcgcggaattaaccacgctcattcctggtacaagcctcacatagaaaccgcgatggaggcaattgctgatactggagcaaactccattcgtgtagttctctcagatggacaacagtggaccaaagatgatgttgacgaagtagcaaaaattatatctttagcagaaaaacattctttagttgctgttcttgaggtacatgatgcactcggaacagatgatattgaaccattacttaaaacagtcgattactggattgagatcaaagatgctttaatcggaaaagaggacaaagtaattattaacatttctaatgaatggtttggttcttggagcagtgaaggttgggcagaaggatataaaaaagcaattcctttactaagagaggcgggtctaaaacatacacttatggttgacgcagctgggtggggacaatttcctagatctattcatgaaaaaggattagacgtttttaactcagacccattaaagaatacaatgttttccattcatatgtatgaatgggcagcgggtaatcctcaacaagtaaaagacaatattgacggtgttcttgaaaagaatttagctgtagtaattggtgagttcggtcatcatcactacggaagagatgttgctgttgatacgatcttaagtcattcagagaagtatgatgtaggttggcttgcctggtcttggcacggaaatagtggtggtgtagagtatcttgacttagcaacagatttttcagggacgcaactaactgaatggggagaaagaattgtgtacggtccgaatggtttaaaagaaacttctgaaatcgttagtgtatacaaaaaataa

SEQ ID NO: 36 - protein, 369 aa, Bacillus alcalophilus
MRSMKLLFAMFILVFSSFTFNLVVAQASGHGQMHKVPWAPQAEAPGKTAENGVWDKVRNNPGKANPPAGKVNGFYIDGTTLYDANGKPFVMRGINHAHSWYKPHIETAMEAIADTGANSIRVVLSDGQQWTKDDVDEVAKIISLAEKHSLVAVLEVHDALGTDDIEPLLKTVDYWIEIKDALIGKEDKVIINISNEWFGSWSSEGWAEGYKKAIPLLREAGLKHTLMVDAAGWGQFPRSIHEKGLDVFNSDPLKNTMFSIHMYEWAAGNPQQVKDNIDGVLEKNLAVVIGEFGHHHYGRDVAVDTILSHSEKYDVGWLAWSWHGNSGGVEYLDLATDFSGTQLTEWGERIVYGPNGLKETSEIVSVYKK

SEQ ID NO: 37 - DNA, 1482 bp, Bacillus sp.
atgaaaaaaaagttatcacagatttatcatttaattatttgcacacttataataagtgtgggaataatggggattacaacgtccccatcagaagcaagttcaggcttttatgttgatggcaatacgttatatgacgcaaacgggcaaccatttgtcatgaaaggcattaaccatggacatgcttggtataaagacaccgcttcaacagctattcctgccattgcagagcaaggcgcgaacacgatacgtattgttttatcagatggcggtcaatgggaaaaagacgacattgacaccgttcgtgaagttattgagcttgcggagcaaaataaaatggtggctgtcgttgaagttcatgatgccacgggccgtgattcacgcagtgatttagatcgggcagtcgattattggatagagatgaaagatgcacttatcggcaaagaggatactgtcattattaacattgcaaacgaatggtatggcagttgggatggcgccgcttgggctgatggctacattgatgtcattccgaagcttcgcgatgccggcttaacacacaccttaatggttgatgcagcaggatgggggcaatatccgcaatctattcatgattacggacaagatgtgtttaatgcagatccgttaaaaaatacgatattctccatccatatgtatgagtatgctggtggtgatgctaacactgttagatcaaatattgatagagtcatagatcaagaccttgctctcgtaataggtgagttcggtcatagacacactgatggcgatgttgatgaagatacaatccttagttattctgaagaaactggcacaggatggctcgcttggtcttggaaaggcaacagtgccgaatgggattatttagacctttcagaagattgggctggtaaccatttaactgattggggaaataggattgtccacggggcaaatggcttgcaggaaacctccaaaccatccaccgtatttacagatgataacggtggtgcccctgaaccgccaactactactaccttgtatgactttgaaggaagcacacaagggtggcatggaagcaacgtgatgggtggcccttggtccgtaacagaatggggtgcgtcaggcaactactctttaaagggcgatgtcaatttaagctcaaattcttcacatgaactgtatagtgaacaaagtcgtaatctacacggatactctcagctaaatgcaaccgttcgccatgccaattggggaaatcccggtaatggcatgaatgcaagactttacgtgaaaacgggctctgattatacatggtatagcggtccttttacacgtatcaatagctccaactcaggtacaacgttatcttttgatttaaacaacatcgaaaatagtcatcatgttagggaaataggtgtgcaattttcagctgcagataatagcagcggtcaaactgctctatacgttgataatgttactttaagataa

SEQ ID NO: 38 - protein, 493 aa, Bacillus sp.
MKKKLSQIYHLIICTLIISVGIMGITTSPSEASSGFYVDGNTLYDANGQPFVMKGINHGHAWYKDTASTAIPAIAEQGANTIRIVLSDGGQWEKDDIDTVREVIELAEQNKMVAVVEVHDATGRDSRSDLDRAVDYWIEMKDALIGKEDTVIINIANEWYGSWDGAAWADGYIDVIPKLRDAGLTHTLMVDAAGWGQYPQSIHDYGQDVFNADPLKNTIFSIHMYEYAGGDANTVRSNIDRVIDQDLALVIGEFGHRHTDGDVDEDTILSYSEETGTGWLAWSWKGNSAEWDYLDLSEDWAGNHLTDWGNRIVHGANGLQETSKPSTVFTDDNGGAPEPPTTTTLYDFEGSTQGWHGSNVMGGPWSVTEWGASGNYSLKGDVNLSSNSSHELYSEQSRNLHGYSQLNATVRHANWGNPGNGMNARLYVKTGSDYTWYSGPFTRINSSNSGTTLSFDLNNIENSHHVREIGVQFSAADNSSGQTALYVDNVTLR

SEQ ID NO: 39 - DNA, 1551 bp, Bacillus circulans
atggggtggtttttagtgattttacgcaagtggttgattgcttttgtcgcatttttactgatgttctcgtggactggacaacttacgaacaaagcacatgctgcaagcggattttatgtaagcggtaccaaattattggatgctacaggacaaccatttgtgatgcgaggagtcaatcatgcgcacacatggtataaagatcaactatccaccgcaataccagccattgctaaaacaggtgccaacacgatacgtattgtactggcgaatggacacaaatggacgcttgatgatgtaaacaccgtcaacaatattctcaccctctgtgaacaaaacaaactaattgccgttttggaagtacatgacgctacaggaagcgatagtctttccgatttagacaacgccgttaattactggattggtattaaaagcgcgttgatcggcaaggaagaccgtgtaatcattaatatagctaacgagtggtacggaacatgggatggagtcgcctgggctaatggttataagcaagccatacccaaactgcgtaatgctggtctaactcatacgctgattgttgactccgctggatggggacaatatccagattcggtcaaaaattatgggacagaagtactgaatgcagacccgttaaaaaacacagtattctctatccatatgtatgaatatgctgggggcaatgcaagtaccgtcaaatccaatattgacggtgtgctgaacaagaatcttgcactgattatcggcgaatttggtggacaacatacaaacggtgatgtggatgaagccaccattatgagttattcccaagagaagggagtcggctggttggcttggtcctggaagggaaatagcagtgatttggcttatctcgatatgacaaatgattgggctggtaactccctcacctcgttcggtaataccgtagtgaatggcagtaacggcattaaagcaacttctgtgttatccggcatttttggaggtgttacgccaacctcaagccctacttctacacctacatctacgccaacctcaactcctactcctacgccaagtccgaccccgagtccaggtaataacgggacgatcttatatgatttcgaaacaggaactcaaggctggtcgggaaacaatatttcgggaggcccatgggtcaccaatgaatggaaagcaacgggagcgcaaactctcaaagccgatgtctccttacaatccaattccacgcatagtctatatataacctctaatcaaaatctgtctggaaaaagcagtctgaaagcaacggttaagcatgcgaactggggcaatatcggcaacgggatttatgcaaaactatacgtaaagaccgggtccgggtggacatggtacgattccggagagaatctgattcagtcaaacgacggtaccattttgacactatccctcagcggcatttcgaatttgtcctcagtcaaagaaattggggtagaattccgcgcctcctcaaacagtagtggccaatcagctatttatgtagatagtgttagtctgcaataa

SEQ ID NO: 40 - protein, 516 aa, Bacillus circulans
MGWFLVILRKWLIAFVAFLLMFSWTGQLTNKAHAASGFYVSGTKLLDATGQPFVMRGVNHAHTWYKDQLSTAIPAIAKTGANTIRIVLANGHKWTLDDVNTVNNILTLCEQNKLIAVLEVHDATGSDSLSDLDNAVNYWIGIKSALIGKEDRVIINIANEWYGTWDGVAWANGYKQAIPKLRNAGLTHTLIVDSAGWGQYPDSVKNYGTEVLNADPLKNTVFSIHMYEYAGGNASTVKSNIDGVLNKNLALIIGEFGGQHTNGDVDEATIMSYSQEKGVGWLAWSWKGNSSDLAYLDMTNDWAGNSLTSFGNTVVNGSNGIKATSVLSGIFGGVTPTSSPTSTPTSTPTSTPTPTPSPTPSPGNNGTILYDFETGTQGWSGNNISGGPWVTNEWKATGAQTLKADVSLQSNSTHSLYITSNQNLSGKSSLKATVKHANWGNIGNGIYAKLYVKTGSGWTWYDSGENLIQSNDGTILTLSLSGISNLSSVKEIGVEFRASSNSSGQSAIYVDSVSLQ

SEQ ID NO: 41 - DNA, 984 bp, Paenibacillus sp.
atgagacaacttttagcaaaaggtattttagctgcactggtcatgatgttagcgatgtatggattggggaatctctcttctaaagcttcggctgcaacaggtttttatgtaagcggtaccactctatatgattctactggtaaaccttttgtaatgcgcggtgtcaatcattcgcatacctggttcaaaaatgatctaaatgcagccatccctgctattgccaaaacaggtgcaaatacagtacgtatcgttttatctaatggtgttcagtatactagagatgatgtaaactcagtcaaaaatattatttccctggttaaccaaaacaaaatgattgctgttcttgaggtgcatgatgctaccggtaaagacgattacgcttctcttgatgccgctgtaaactactggatcagcatcaaagatgccttgattggcaaggaagatcgagtcattgttaatattgccaatgaatggtacggtacatggaatggcagtgcttgggcagatggttataagcaggctattcccaaactaagaaatgcaggcatcaaaaacactttaatcgttgatgccgccggctggggacaatgtcctcaatcgatcgttgattacgggcaaagtgtatttgcagcagattcgcttaaaaatacaattttctctattcacatgtatgaatatgcaggcggtacagatgcgatcgtcaaaagcaatatggaaaatgtactgaacaaaggacttcctttgatcatcggtgaatttggcgggcagcatacaaacggcgatgtagatgaacatgcaattatgcgttatggtcagcaaaaaggtgtaggttggctggcatggtcgtggtatggcaacaatagtgaactcagttatctggatttggctacaggtcccgccggtagtctgacaagtatcggcaatacgattgtaaatgatccatatggtatcaaagctacctcgaaaaaagcgggtatcttctaa

SEQ ID NO: 42 - protein, 327 aa, Paenibacillus sp.
MRQLLAKGILAALVMMLAMYGLGNLSSKASAATGFYVSGTTLYDSTGKPFVMRGVNHSHTWFKNDLNAAIPAIAKTGANTVRIVLSNGVQYTRDDVNSVKNIISLVNQNKMIAVLEVHDATGKDDYASLDAAVNYWISIKDALIGKEDRVIVNIANEWYGTWNGSAWADGYKQAIPKLRNAGIKNTLIVDAAGWGQCPQSIVDYGQSVFAADSLKNTIFSIHMYEYAGGTDAIVKSNMENVLNKGLPLIIGEFGGQHTNGDVDEHAIMRYGQQKGVGWLAWSWYGNNSELSYLDLATGPAGSLTSIGNTIVNDPYGIKATSKKAGIF

SEQ ID NO: 43 - DNA, 981 bp, Bacillus circulans
atggccaagttgcaaaagggtacaatcttaacagtcattgcagcactgatgtttgtcattttggggagcgcggcgcccaaagccgcagcagctacaggtttttacgtgaatggaggcaaattgtacgattctacgggtaaaccattttacatgaggggtatcaatcatgggcactcctggtttaaaaatgatttgaacacggctatccctgcgatcgcaaaaacgggtgccaatacggtacgaattgttttatcaaacggtacacaatacaccaaggatgatctgaattccgtaaaaaacatcattaatgtcgtaaatgcaaacaagatgattgctgtgcttgaagtacacgatgccactgggaaagatgacttcaactcgttggatgcagcggtcaactactggataagcatcaaagaagcactgatcgggaaggaagatcgggttattgtaaacattgcaaacgagtggtacggaacatggaacggaagcgcgtgggctgacgggtacaaaaaagctattccgaaattaagagatgcgggtattaaaaataccttgattgtagatgcagcaggctggggtcagtaccctcaatcgatcgtcgattacggacaaagcgtattcgccgcggattcacagaaaaatacggcgttttccattcacatgtatgagtatgcaggcaaggatgcggccaccgtcaaatccaatatggaaaatgtgctgaataaggggctggccttaatcattggtgagttcggaggatatcacaccaatggagatgtcgatgaatatgcaatcatgaaatatggtctggaaaaaggggtaggatggcttgcatggtcttggtacggtaatagctctggattaaactatcttgatttggcaacaggacctaacggcagtttgacgagctatggtaatacggttgtcaatgatacttacggaattaaaaatacgtcccaaaaagcgggaatcttttaa

SEQ ID NO: 44 - protein, 326 aa, Bacillus circulans
MAKLQKGTILTVIAALMFVILGSAAPKAAAATGFYVNGGKLYDSTGKPFYMRGINHGHSWFKNDLNTAIPAIAKTGANTVRIVLSNGTQYTKDDLNSVKNIINVVNANKMIAVLEVHDATGKDDFNSLDAAVNYWISIKEALIGKEDRVIVNIANEWYGTWNGSAWADGYKKAIPKLRDAGIKNTLIVDAAGWGQYPQSIVDYGQSVFAADSQKNTAFSIHMYEYAGKDAATVKSNMENVLNKGLALIIGEFGGYHTNGDVDEYAIMKYGLEKGVGWLAWSWYGNSSGLNYLDLATGPNGSLTSYGNTVVNDTYGIKNTSQKAGIF

SEQ ID NO: 45 - DNA, 1110 bp, Bacillus nealsonii
atggttgtgaaaaaattatcaagttttattctaattttactgttagttacttctgctttgtttattactgattcaaaagcaagtgctgcttcgggattttatgtaagcggtaccactttatatgatgcaacgggtaaaccgtttactatgagaggtgtaaatcatgctcattcttggtttaaagaagattcagcagctgctattccagcaatagcagcaactggagcaaacacagtaagaattgttttatctgatggtggacaatacaccaaagatgatattaatactgttaaaagccttttgtcattggcagaaaaaataaacttgcattctggagtcatgacgcacagaaaagacgatgtggaatctttaaatcgtgcagtcgattattggatcagcttaaaagacacattgataggcaaagaagataaagtgataataaacattgcgaatgaatggtatggtacttgggatggtgcggcatgggcagctggttataaacaagctattccaaagttacggaatgcaggcttaaatcatactctaataattgattctgctggatggggacaatacccagcttccattcataattatggaaaagaggtatttaatgcggatccattgaaaaatacaatgttctccatacatatgtatgagtacgctggtggggatgcagcaactgttaagtcaaatattgatggtgtcttaaaccaaggattagctttaataataggagagtttggacaaaaacatacaaatggagatgtagatgaagcaaccatcatgagttattcacagcaaaaaaatatcggttggcttgcatggtcttggaaaggaaatagcacagattggagctatctggatttaagcaacgattggtctggtaacagtttaactgattggggtaatacggttgttaatggggcaaatgggttaaaagccacttcaaaactaagcggagtattcggtagctcagcaggaacaaataatatattgtatgattttgaaagcggtaatcaaaactggactggatcaaatatcgcgggtggaccttggaacgaattcaagcttgatatcattcaggacgagcctcagactccagcgtaa

SEQ ID NO: 46 - protein, 369 aa, Bacillus nealsonii
MVVKKLSSFILILLLVTSALFITDSKASAASGFYVSGTTLYDATGKPFTMRGVNHAHSWFKEDSAAAIPAIAATGANTVRIVLSDGGQYTKDDINTVKSLLSLAEKINLHSGVMTHRKDDVESLNRAVDYWISLKDTLIGKEDKVIINIANEWYGTWDGAAWAAGYKQAIPKLRNAGLNHTLIIDSAGWGQYPASIHNYGKEVFNADPLKNTMFSIHMYEYAGGDAATVKSNIDGVLNQGLALIIGEFGQKHTNGDVDEATIMSYSQQKNIGWLAWSWKGNSTDWSYLDLSNDWSGNSLTDWGNTVVNGANGLKATSKLSGVFGSSAGTNNILYDFESGNQNWTGSNIAGGPWNEFKLDIIQDEPQTPA

SEQ ID NO: 47 - DNA, 984 bp, Bacillus circulans
atgatgttgatatggatgcagggatggaagtctattctagtcgcgatcttggcgtgtgtgtcagtaggcggtgggcttcctagtccagaagcagccacaggattttatgtaaacggtaccaagctgtatgattcaacgggcaaggcctttgtgatgaggggtgtaaatcatccccacacctggtacaagaatgatctgaacgcggctattccggctatcgcgcaaacgggagccaataccgtacgagtcgtcttgtcgaacgggtcgcaatggaccaaggatgacctgaactccgtcaacagtatcatctcgctggtgtcgcagcatcaaatgatagccgttctggaggtgcatgatgcgacaggcaaagatgagtatgcttcccttgaagcggccgtcgactattggatcagcatcaaaggggcattgatcggaaaagaagaccgcgtcatcgtcaatattgctaatgaatggtatggaaattggaacagcagcggatgggccgatggttataagcaggccattcccaaattaagaaacgcgggcattaagaatacgttgatcgttgatgcagcgggatgggggcaatacccgcaatccatcgtggatgagggggccgcggtatttgcttccgatcaactgaagaatacggtattctccatccatatgtatgagtatgccggtaaggatgccgctacggtgaaaacgaatatggacgatgttttaaacaaaggattgcctttaatcattggggagttcggcggctatcatcaaggtgccgatgtcgatgagattgctattatgaagtacggacagcagaaggaagtgggctggctggcttggtcctggtacggaaacagcccggagctgaacgatttggatctggctgcagggccaagcggaaacctgaccggctggggaaacacggtggttcatggaaccgacgggattcagcaaacctccaagaaagcgggcatttattaa

SEQ ID NO: 48 - protein, 327 aa, Bacillus circulans
MMLIWMQGWKSILVAILACVSVGGGLPSPEAATGFYVNGTKLYDSTGKAFVMRGVNHPHTWYKNDLNAAIPAIAQTGANTVRVVLSNGSQWTKDDLNSVNSIISLVSQHQMIAVLEVHDATGKDEYASLEAAVDYWISIKGALIGKEDRVIVNIANEWYGNWNSSGWADGYKQAIPKLRNAGIKNTLIVDAAGWGQYPQSIVDEGAAVFASDQLKNTVFSIHMYEYAGKDAATVKTNMDDVLNKGLPLIIGEFGGYHQGADVDEIAIMKYGQQKEVGWLAWSWYGNSPELNDLDLAAGPSGNLTGWGNTVVHGTDGIQQTSKKAGIY